European Patent Application EP 4 785 951 A1, published August 5, 2026. Title: 非洲猪瘟病毒免疫原组合及其应用. Applicant: 复旦大学附属中山医院. Application CN. The sequence listing filed with the application follows.

SEQUENCE LISTING (100 sequences)

SEQ ID NO: 1 - DNA, 1941 bp, African Swine fever virus
  source 1..1941: mol_type = genomic DNA
atggcatcaggaggagctttttgtcttattgctaacgatgggaaggccgacaagattatattggcccaagacttgctgaatagcaggatctctaacattaaaaatgtgaacaaaagttatgggaaacccgatcccgaacccactttgagtcaaatcgaagaaacacatttggtgcattttaatgcgcattttaagccttatgttccagtagggtttgaatacaataaagtacgcccgcatacgggtacccccaccttgggaaacaagcttacctttggtattccccagtacggagactttttccatgatatggtgggccatcatatattgggtgcatgtcattcatcctggcaggatgctccgattcagggcacgtcccagatgggggcccatgggcagcttcaaacgtttcctcgcaacggatatgactgggacaaccaaacacccttagagggcgccgtttacacgcttgtagatccttttggaagacccattgtacccggcacaaagaatgcgtaccgaaacttggtttactactgcgaataccccggagaacgactttatgaaaacgtaagattcgatgtaaatggaaattccctagacgaatatagttcggatgtcacaacgcttgtgcgcaaattttgcatcccaggggataaaatgactggatataagcacttggttggccaggaggtatcggtggagggaaccagtggccctctcctatgcaacattcatgatttgcacaagccgcaccaaagcaaacctattcttaccgatgaaaatgatacgcagcgaacgtgtagccataccaacccgaaatttctttcacagcattttcccgagaactctcacaatatccaaacagcaggtaaacaagatattactcctatcacggacgcaacgtatctggacataagacgtaatgttcattacagctgtaatggacctcaaacccctaaatactatcagccccctcttgcgctctggattaagttgcgcttttggtttaatgagaacgtgaaccttgctattccctcagtatccattcccttcggcgagcgctttatcaccataaagcttgcatcgcaaaaggatttggtgaatgaatttcctggactttttgtacgccagtcacgttttatagctggacgccccagtagacgcaatatacgctttaaaccatggtttatcccaggagtcattaatgaaatctcgctcacgaataatgaactttacatcaataacctgtttgtaacccctgaaatacacaacctttttgtaaaacgcgttcgcttttcgctgatacgtgtccataaaacgcaggtgacccacaccaacaataaccaccacgatgaaaaactaatgtctgctcttaaatggcccattgaatatatgtttataggattaaaacctacctggaacatctccgatcaaaatcctcatcaacaccgagattggcacaagttcggacatgttgttaacgccattatgcagcccactcaccacgcagagataagctttcaggatagagatacagctcttccagacgcatgttcatctatatctgatattagccccgttacgtatccgatcacattacctattattaaaaacatttccgtaactgctcatggtatcaatcttatcgataaatttccatcaaagttctgcagctcttacatacccttccactacggaggcaatgcgattaaaacccccgatgatccgggtgcgatgatgattacctttgctttgaagccacgggaggaataccaacccagtggtcatattaacgtatccagagcaagagaattttatattagttgggacacggattacgtggggtctatcactacggctgatcttgtggtatcggcatctgctattaactttcttcttcttcagaacggttcagctgtgctgcgttacagtacctaa

SEQ ID NO: 2 - protein, 646 aa, African Swine fever virus
MASGGAFCLIANDGKADKIILAQDLLNSRISNIKNVNKSYGKPDPEPTLSQIEETHLVHFNAHFKPYVPVGFEYNKVRPHTGTPTLGNKLTFGIPQYGDFFHDMVGHHILGACHSSWQDAPIQGTSQMGAHGQLQTFPRNGYDWDNQTPLEGAVYTLVDPFGRPIVPGTKNAYRNLVYYCEYPGERLYENVRFDVNGNSLDEYSSDVTTLVRKFCIPGDKMTGYKHLVGQEVSVEGTSGPLLCNIHDLHKPHQSKPILTDENDTQRTCSHTNPKFLSQHFPENSHNIQTAGKQDITPITDATYLDIRRNVHYSCNGPQTPKYYQPPLALWIKLRFWFNENVNLAIPSVSIPFGERFITIKLASQKDLVNEFPGLFVRQSRFIAGRPSRRNIRFKPWFIPGVINEISLTNNELYINNLFVTPEIHNLFVKRVRFSLIRVHKTQVTHTNNNHHDEKLMSALKWPIEYMFIGLKPTWNISDQNPHQHRDWHKFGHVVNAIMQPTHHAEISFQDRDTALPDACSSISDISPVTYPITLPIIKNISVTAHGINLIDKFPSKFCSSYIPFHYGGNAIKTPDDPGAMMITFALKPREEYQPSGHINVSRAREFYISWDTDYVGSITTADLVVSASAINFLLLQNGSAVLRYST

SEQ ID NO: 3 - DNA, 1593 bp, African Swine fever virus
  source 1..1593: mol_type = genomic DNA
atggcagaatttaatattgatgagcttctcaaaaacgtattggaggatccctctactgaaatatccgaagaaacgcttaaacagctttaccaaaggacgaacccttacaaacagttcaaaaatgatagcagggtggccttttgctcttttacaaatttgcgggagcagtatattcgacgtcttataatgactagctttattggatatgtcttcaaagctctgcaggaatggatgccttcctattcaaaacctacccacacgaccaaaactcttctcagtgagctaataacgttagttgatactttgaaacaggaaactaatgatgttccctctgaatcggtagtaaatacaattttatctatagcagatagctgcaaaacccagacgcagaaaagcaaggaagctaaaacaacgatcgatagctttttacgagaacattttgtgtttgatcctaatcttcatgctcaaagtgcgtatacttgtgcagataccaatgtagacacttgtgcaagcatgtgtgcagataccaatgtagacacctgtgcaagcatgtgtgcagataccaatgtagatacctgtgcaagcacttgtacaagcacagaatacaccgatttagcagatcctgagcgcatccctttacacatcatgcaaaaaacattaaatgtgcctaatgagcttcaggccgatattgatgcaatcacccaaaccccacagggctatagggcagcagcccacatattacaaaatatagaacttcaccaaagcattaaacatatgcttgaaaatccgagggcgtttaaacccattctctttaacacaaaaattactagatatctttcgcagcatattccacctcaggatactttttataagtggaattattacattgaggataattacgaagagttgcgggccgctacggaaagcatctacccagaaaaacccgacctagagtttgccttcattatttatgatgtggtggatagcagcaaccaacaaaaggttgatgaattttattataaatataaagaccagattttctcagaggtttcatccattcaattaggcaactggacactcctgggaagctttaaggccaacagagagcgctacaattattttaatcaaaataatgaaataataaaacggattttggaccgtcatgaggaagacctaaagataggaaaagagattttacgaaatactatttaccacaaaaaagcaaaaaatatacaagaaactggcccggatgctccggggctctccatctataattcaacctttcacacggatagcgggattaagggactgctttcctttaaggagctaaaaaacctagaaaaagcatctggaaatatcaaaaaagctcgagagtatgattttatagacgactgcgaagaaaaaattaagcaactgcttagtaaagaaaatttaacccccgatgaagaaagcgagctgataaaaacaaaaaaacagttagataatgcgcttgaaatgctcaatgtgcctgatgatacgatacgggtagatatgtgggtcaacaataataataaactcgaaaaagaaattttatatacaaaagcagaattgtaa

SEQ ID NO: 4 - protein, 530 aa, African Swine fever virus
MAEFNIDELLKNVLEDPSTEISEETLKQLYQRTNPYKQFKNDSRVAFCSFTNLREQYIRRLIMTSFIGYVFKALQEWMPSYSKPTHTTKTLLSELITLVDTLKQETNDVPSESVVNTILSIADSCKTQTQKSKEAKTTIDSFLREHFVFDPNLHAQSAYTCADTNVDTCASMCADTNVDTCASMCADTNVDTCASTCTSTEYTDLADPERIPLHIMQKTLNVPNELQADIDAITQTPQGYRAAAHILQNIELHQSIKHMLENPRAFKPILFNTKITRYLSQHIPPQDTFYKWNYYIEDNYEELRAATESIYPEKPDLEFAFIIYDVVDSSNQQKVDEFYYKYKDQIFSEVSSIQLGNWTLLGSFKANRERYNYFNQNNEIIKRILDRHEEDLKIGKEILRNTIYHKKAKNIQETGPDAPGLSIYNSTFHTDSGIKGLLSFKELKNLEKASGNIKKAREYDFIDDCEEKIKQLLSKENLTPDEESELIKTKKQLDNALEMLNVPDDTIRVDMWVNNNNKLEKEILYTKAEL

SEQ ID NO: 5 - DNA, 726 bp, African Swine fever virus
  source 1..726: mol_type = genomic DNA
atggctgcaaacattattgcaacaagagccgtgccaaagatggccagcaaaaaagagcatcaatactgtctgctagactcccaggaaaagcgtcatgggcattatcccttttcatttgaattaaagccttatgggcaaacaggcgcaaatatcataggagtacagggctcacttacccatgttatcaaaatgacagtatttccatttatgattccttttcctttacaaaaaactcatatagatgattttattggtggacgcatttatttattttttaaggaactggacatgcaagcagtttctgatgtaaatggaatgcaataccacttcgagttcaaggttgttcctgtaagccccaaccaagtagagcttcttcctgtgaataataaatataaatttacatatgctataccggtagtgcaataccttaccccaatcttttatgatctttcgggaccgctagatttcccattagatactctttcggtccatgtggatatcctctccaatcatatacagcttcctatccaaaaccataacctaacaacgggtgatcgtgtttttatttctggatataaacacctgcaaacgattgaattatgtaaaaataacaagatttttatcaaaaatataccgccgctttcatccgaaaaaataaaactatatatactaaaaaatcgaatcagaattccgctatactttaaatctttaaaaacgtctaagtaa

SEQ ID NO: 6 - protein, 241 aa, African Swine fever virus
MAANIIATRAVPKMASKKEHQYCLLDSQEKRHGHYPFSFELKPYGQTGANIIGVQGSLTHVIKMTVFPFMIPFPLQKTHIDDFIGGRIYLFFKELDMQAVSDVNGMQYHFEFKVVPVSPNQVELLPVNNKYKFTYAIPVVQYLTPIFYDLSGPLDFPLDTLSVHVDILSNHIQLPIQNHNLTTGDRVFISGYKHLQTIELCKNNKIFIKNIPPLSSEKIKLYILKNRIRIPLYFKSLKTSK

SEQ ID NO: 7 - DNA, 1317 bp, African Swine fever virus
  source 1..1317: mol_type = genomic DNA
atgtatcatgattatgcttcaaagctgttagccgattataggtcagatccacctctttgggaaagcgatttgccgcgtcataaccggtattctgataatatactaaattcccggtactgcggcaacaaaaatggagctgcgcctgtatacaatgaatacactaatagtcctgaaaaggctgaaaagggattgcaactcagtgatctacgtaacttttcttttatgctgaaccctcagcacaaaaacattggttacggcgatgcgcaagatctggagccgtacagctccattccaaaaaataaactttttaatcattttaaaaatcatcgtcctgctttttcaacccatacggaaaacctaattaggcgcaatgttgttcgtacggaaaaaaaaacatttccgcaggtggctagcttaaagggcacacagaaaaattgtctgacccagccttcctcattgccttccttaaaaaacccaaaaaatagttcggttccttctacgaggttcagcgagcacacaaaatttttttcgtacgaggatcttcctaaactcagaacaaagggtaccattaagcatgagcagcaccttggcgatcagatgccgggccagcactataacggatatattccgcacaaagacgtgtacaatattttgtgtttagcgcacaatctacctgcgtcggtagaaaaagggattgcaggtagaggtattcctttaggaaatccacatgtcaaaccgaacatagagcaggaactcataaaatccaccagtacctacacggacgtgccgatgcttggtccccttccgcccaaagattcgcaacacggcagagaataccaggaattttccgcaaatagacatatgctacaagtatctaatatactacattctgtgtttgctaatcattctataaagccacaaatcctagaagacataccggtactcaatgcacaactaacaagcataaagccggtaagcccatttttaaacaaagcgtatcaaacccattatatggaaaatattgttaccttggtgccccggtttaagagtattgccaactactcaagccctataccgaattattctaaaagaaatagcggtcaggctgaatattttgatacctcaaagcaaacaatttcaagacacaataattatatacctaaatatacgggaggaattggagattccaaactagacagcacctttcctaaagatttcaacgcctcctcggtaccgttaacaagcgcggaaaaggaccattccctgcggggagacaactcagcatgttgcatctcatctatatctccatcattgtga

SEQ ID NO: 8 - protein, 438 aa, African Swine fever virus
MYHDYASKLLADYRSDPPLWESDLPRHNRYSDNILNSRYCGNKNGAAPVYNEYTNSPEKAEKGLQLSDLRNFSFMLNPQHKNIGYGDAQDLEPYSSIPKNKLFNHFKNHRPAFSTHTENLIRRNVVRTEKKTFPQVASLKGTQKNCLTQPSSLPSLKNPKNSSVPSTRFSEHTKFFSYEDLPKLRTKGTIKHEQHLGDQMPGQHYNGYIPHKDVYNILCLAHNLPASVEKGIAGRGIPLGNPHVKPNIEQELIKSTSTYTDVPMLGPLPPKDSQHGREYQEFSANRHMLQVSNILHSVFANHSIKPQILEDIPVLNAQLTSIKPVSPFLNKAYQTHYMENIVTLVPRFKSIANYSSPIPNYSKRNSGQAEYFDTSKQTISRHNNYIPKYTGGIGDSKLDSTFPKDFNASSVPLTSAEKDHSLRGDNSACCISSISPSL

SEQ ID NO: 9 - DNA, 585 bp, African Swine fever virus
  source 1..585: mol_type = genomic DNA
atggattttattttaaatatatccatgaaaatggaggtcatcttcaaaacggatttaagatcatcttcacaagttgtgtttcatgcgggtagcctgtataattggttttctgttgagattatcaatagcggtagaattgttacgaccgctataaaaacattgcttagtactgttaagtatgatattgtgaaatctgctcgtatatatgcagggcaagggtatactgaacatcaggctcaagaagaatggaatatgattctgcatgtgctgtttgaagaggagacggaatcctcagcatcttcggagaacattcatgaaaaaaatgataatgaaaccaatgaatgcacatcctcctttgaaacgttgtttgagcaagagccctcatcggaggtacctaaagactccaagctgtatatgcttgcacaaaagactgtgcaacatattgaacaatatggaaaggcacctgattttaacaaggttattagagcacataattttattcaaaccatttatggaacccctctaaaggaagaagaaaaagaggtggtaagactcatggttattaaacttttaaaaaaaaaataa

SEQ ID NO: 10 - protein, 194 aa, African Swine fever virus
MDFILNISMKMEVIFKTDLRSSSQVVFHAGSLYNWFSVEIINSGRIVTTAIKTLLSTVKYDIVKSARIYAGQGYTEHQAQEEWNMILHVLFEEETESSASSENIHEKNDNETNECTSSFETLFEQEPSSEVPKDSKLYMLAQKTVQHIEQYGKAPDFNKVIRAHNFIQTIYGTPLKEEEKEVVRLMVIKLLKKK

SEQ ID NO: 11 - DNA, 354 bp, African Swine fever virus
  source 1..354: mol_type = genomic DNA
atggacactgaaacgtctccactgctttctcataacctgtcaacccgcgagggaattaaacaaagcacccaaggccttttagcccatacaatcgccaaatatcccggaacaactgcgattctcctgggcattttgattttgctcattattattcttatcatcgttgccatcgtttactataaccggactattgactgcaagtcgagcatacctaaacctcctcctagctactatgtacaacaacctgagcctcaccaccatttcccggtattctttagaaaaaggaaaaactccacctccctgcagtcccacattccaagcgacgaacaattagctgaacttgcgcattcatga

SEQ ID NO: 12 - protein, 117 aa, African Swine fever virus
MDTETSPLLSHNLSTREGIKQSTQGLLAHTIAKYPGTTAILLGILILLIIILIIVAIVYYNRTIDCKSSIPKPPPSYYVQQPEPHHHFPVFFRKRKNSTSLQSHIPSDEQLAELAHS

SEQ ID NO: 13 - DNA, 555 bp, African Swine fever virus
  source 1..555: mol_type = genomic DNA
atggattctgaattttttcaaccggtttatccgcggcattatggtgagtgtttgtcaccagtcactacaccaagcttcttctccacacatatgtatactattctcattgctatcgtggtcttagtcatcattatcatcgttctaatctatctattctcttcaagaaagaaaaaagctgctgctattgaggaggaagatatacagtttataaatccttatcaagatcagcagtgggtagaagtcactccacaaccaggtacctctaaaccagctggagcgactacagcaagtgtaggcaagccagtcacgggcagaccggcaacaaacagaccagcaacaaacaaaccagttacggacaacccagttacggacagactagtcatggcaactggcgggccggcggccgcacctgcggccgcgagtgctcctgctcatccggctgagccttacacgacagtcactactcagaacactgcttcacaaacaatgtcggctattgaaaatttacgacaaagaaacacctatacgcataaagacctagaaaactccttgtaa

SEQ ID NO: 14 - protein, 184 aa, African Swine fever virus
MDSEFFQPVYPRHYGECLSPVTTPSFFSTHMYTILIAIVVLVIIIIVLIYLFSSRKKKAAAIEEEDIQFINPYQDQQWVEVTPQPGTSKPAGATTASVGKPVTGRPATNRPATNKPVTDNPVTDRLVMATGGPAAAPAAASAPAHPAEPYTTVTTQNTASQTMSAIENLRQRNTYTHKDLENSL

SEQ ID NO: 15 - DNA, 63 bp, African Swine fever virus
  source 1..63: mol_type = genomic DNA
tttatgcgcgaaattaaagtaaaggaagtgttatacttttatacaatgcaggctgcccaagag

SEQ ID NO: 16 - protein, 21 aa, African Swine fever virus
FMREIKVKEVLYFYTMQAAQE

SEQ ID NO: 17 - DNA, 129 bp, African Swine fever virus
  source 1..129: mol_type = genomic DNA
ggaagagttcccggtttttcaaaagaaatgctatttcaatatatacgctactttacagataatttgtgcttcatgatgcagtgcaaaagcatttataaggtgggaaacccttttcctcagatgactaaa

SEQ ID NO: 18 - protein, 43 aa, African Swine fever virus
GRVPGFSKEMLFQYIRYFTDNLCFMMQCKSIYKVGNPFPQMTK

SEQ ID NO: 19 - DNA, 99 bp, African Swine fever virus
  source 1..99: mol_type = genomic DNA
acggaacaatttattagaaaccgcattaatttcattccgatttatgcgaaaaacgagacactggtatttgctctgcggagtttaaacaatagctgtgag

SEQ ID NO: 20 - protein, 33 aa, African Swine fever virus
TEQFIRNRINFIPIYAKNETLVFALRSLNNSCE

SEQ ID NO: 21 - DNA, 69 bp, African Swine fever virus
  source 1..69: mol_type = genomic DNA
attgaacagtacccaacggataaaaaagaatatatggcgcttagcggttacaagcaaagctctatgacc

SEQ ID NO: 22 - protein, 23 aa, African Swine fever virus
IEQYPTDKKEYMALSGYKQSSMT

SEQ ID NO: 23 - DNA, 93 bp, African Swine fever virus
  source 1..93: mol_type = genomic DNA
caaaataaccaaatagaaactattctggttcaaaaacgttacagccttgctttttcagaatttattcattgtcattactctataaatgctaat

SEQ ID NO: 24 - protein, 31 aa, African Swine fever virus
QNNQIETILVQKRYSLAFSEFIHCHYSINAN

SEQ ID NO: 25 - DNA, 78 bp, African Swine fever virus
  source 1..78: mol_type = genomic DNA
gaccgcatgtggtatcatatttggattgaaactccagtctacgaactataccacaaaaaataccaaaaatttaggaaa

SEQ ID NO: 26 - protein, 26 aa, African Swine fever virus
DRMWYHIWIETPVYELYHKKYQKFRK

SEQ ID NO: 27 - DNA, 90 bp, African Swine fever virus
  source 1..90: mol_type = genomic DNA
tttaaaaaatctatgtcatactttgacggtaaaacagaatataagcatatctacttccttgcaatgttatgtaagtcgttggaggaaccc

SEQ ID NO: 28 - protein, 30 aa, African Swine fever virus
FKKSMSYFDGKTEYKHIYFLAMLCKSLEEP

SEQ ID NO: 29 - DNA, 99 bp, African Swine fever virus
  source 1..99: mol_type = genomic DNA
gtggcccaaggtgaccatgtgcctgaccatatcaacatcctaaaaagaaaccaaatatttccgctgtttgcgcctaccccaagaggcgagggtagattt

SEQ ID NO: 30 - protein, 33 aa, African Swine fever virus
VAQGDHVPDHINILKRNQIFPLFAPTPRGEGRF

SEQ ID NO: 31 - DNA, 102 bp, African Swine fever virus
  source 1..102: mol_type = genomic DNA
aatagcggaagaggatatatgcatgtaagattttctgctgttgtttcttacttaaatgcctttgatttaatagcggccgttaaaattattaaaaatgacagt

SEQ ID NO: 32 - protein, 34 aa, African Swine fever virus
NSGRGYMHVRFSAVVSYLNAFDLIAAVKIIKNDS

SEQ ID NO: 33 - DNA, 87 bp, African Swine fever virus
  source 1..87: mol_type = genomic DNA
tcgcaaaataatgttgcagaagtggggcaaattgtgccggtacagcttgctaacagcagcgtgtactatatacctggcagacaacag

SEQ ID NO: 34 - protein, 29 aa, African Swine fever virus
SQNNVAEVGQIVPVQLANSSVYYIPGRQQ

SEQ ID NO: 35 - DNA, 69 bp, African Swine fever virus
  source 1..69: mol_type = genomic DNA
tctaaaaaagacttcaagcagatatgcttttttgaaaaactttactatacctactctataagctcggat

SEQ ID NO: 36 - protein, 23 aa, African Swine fever virus
SKKDFKQICFFEKLYYTYSISSD

SEQ ID NO: 37 - DNA, 81 bp, African Swine fever virus
  source 1..81: mol_type = genomic DNA
atgataattaacgtcatcatggatgtattttacgagacatattctttaccttataacatcaatctaacccgtgaacaaatt

SEQ ID NO: 38 - protein, 27 aa, African Swine fever virus
MIINVIMDVFYETYSLPYNINLTREQI

SEQ ID NO: 39 - DNA, 81 bp, African Swine fever virus
  source 1..81: mol_type = genomic DNA
ggattaaataaaaagcgagaacttaaatactcctttcatatcatactttatacatactcagtattaaacaataatgaggcc

SEQ ID NO: 40 - protein, 27 aa, African Swine fever virus
GLNKKRELKYSFHIILYTYSVLNNNEA

SEQ ID NO: 41 - DNA, 72 bp, African Swine fever virus
  source 1..72: mol_type = genomic DNA
gaccaagtgatgacaaagagcatagaggttcatgagtccattctctttgaagaactgcctgatactcaaaaa

SEQ ID NO: 42 - protein, 24 aa, African Swine fever virus
DQVMTKSIEVHESILFEELPDTQK

SEQ ID NO: 43 - DNA, 99 bp, African Swine fever virus
  source 1..99: mol_type = genomic DNA
gaatcgatttttaatcaattcaatagcggcctgcacaaatactttgctccctcttttgccattttcatgtggatgctcgaaacggcaaattatgttata

SEQ ID NO: 44 - protein, 33 aa, African Swine fever virus
ESIFNQFNSGLHKYFAPSFAIFMWMLETANYVI

SEQ ID NO: 45 - DNA, 66 bp, African Swine fever virus
  source 1..66: mol_type = genomic DNA
tgcttggacgcaaacctaggaaatcgaacgtataatattctacagcgttttcgcggggatgtccct

SEQ ID NO: 46 - protein, 22 aa, African Swine fever virus
CLDANLGNRTYNILQRFRGDVP

SEQ ID NO: 47 - DNA, 105 bp, African Swine fever virus
  source 1..105: mol_type = genomic DNA
ttgaccaatgaacaattaatgacgaaactcgttgatgaatttgttcagtatgatttaagcgcgatcagctttgagtttaagcttaaaaagcccaataaaacggac

SEQ ID NO: 48 - protein, 35 aa, African Swine fever virus
LTNEQLMTKLVDEFVQYDLSAISFEFKLKKPNKTD

SEQ ID NO: 49 - DNA, 84 bp, African Swine fever virus
  source 1..84: mol_type = genomic DNA
attgatattcatgaagtacgatatggagcctacacacttttcatgtatggttccctcgaaaacggttacaaagcagaagtaagg

SEQ ID NO: 50 - protein, 28 aa, African Swine fever virus
IDIHEVRYGAYTLFMYGSLENGYKAEVR

SEQ ID NO: 51 - DNA, 123 bp, African Swine fever virus
  source 1..123: mol_type = genomic DNA
atggggtaccgcgagaaggaaaaagagtttgcaccatacattcgaatattttttaaaagcctgtatgagcgacgaaaagccattacttacttaaataatatgggctacaacacggccgcggac

SEQ ID NO: 52 - protein, 41 aa, African Swine fever virus
MGYREKEKEFAPYIRIFFKSLYERRKAITYLNNMGYNTAAD

SEQ ID NO: 53 - DNA, 75 bp, African Swine fever virus
  source 1..75: mol_type = genomic DNA
tcccgagaattaaaactacctcttacaagttggatacagcttcagcactattcctacgagcctcgcggcttggta

SEQ ID NO: 54 - protein, 25 aa, African Swine fever virus
SRELKLPLTSWIQLQHYSYEPRGLV

SEQ ID NO: 55 - DNA, 141 bp, African Swine fever virus
  source 1..141: mol_type = genomic DNA
aatgttatccccgatcgcagagaggtaggaattctgtcatacacctcgctgtatgactgtatctactacgcgggaggacacaaggtatgcaatatgctcattgcctatgccatccatgatgaatacggccgtattgcttgc

SEQ ID NO: 56 - protein, 47 aa, African Swine fever virus
NVIPDRREVGILSYTSLYDCIYYAGGHKVCNMLIAYAIHDEYGRIAC

SEQ ID NO: 57 - DNA, 78 bp, African Swine fever virus
  source 1..78: mol_type = genomic DNA
cgggatgaggcaaatagcctcatggccaagggtgaatctcttcactacgtctcctttcactttaacaatcgtctcgtg

SEQ ID NO: 58 - protein, 26 aa, African Swine fever virus
RDEANSLMAKGESLHYVSFHFNNRLV

SEQ ID NO: 59 - DNA, 69 bp, African Swine fever virus
  source 1..69: mol_type = genomic DNA
cacgaaaaagtgcttctgtctatgaaagccatgtctacactatgcgccgaggtgaatgaatacctgcga

SEQ ID NO: 60 - protein, 23 aa, African Swine fever virus
HEKVLLSMKAMSTLCAEVNEYLR

SEQ ID NO: 61 - DNA, 63 bp, African Swine fever virus
  source 1..63: mol_type = genomic DNA
atggtgttaatagagtttttaacaggtttcttctatttatatggaaagagactgttttccatt

SEQ ID NO: 62 - protein, 21 aa, African Swine fever virus
MVLIEFLTGFFYLYGKRLFSI

SEQ ID NO: 63 - DNA, 90 bp, African Swine fever virus
  source 1..90: mol_type = genomic DNA
tgtcggaagaacattttcttccttccaaatgattttagcaagcataccctacaatggctgggattatattggaaagagcatggctccgtc

SEQ ID NO: 64 - protein, 30 aa, African Swine fever virus
CRKNIFFLPNDFSKHTLQWLGLYWKEHGSV

SEQ ID NO: 65 - DNA, 87 bp, African Swine fever virus
  source 1..87: mol_type = genomic DNA
ctggccgtgaaaaatcaatcttccaggaaaactttgaacttgttgctatcttacataaattacaaggtgaaaaatgttaaaaagctg

SEQ ID NO: 66 - protein, 29 aa, African Swine fever virus
LAVKNQSSRKTLNLLLSYINYKVKNVKKL

SEQ ID NO: 67 - DNA, 126 bp, African Swine fever virus
  source 1..126: mol_type = genomic DNA
acagaaagaattacttatctcaaacagatagtgcacaccataaaatatgaaagtggaaggcgatttttggtagacatcattcacagcatttaccaaagttactcactaaaacacgaagatattctt

SEQ ID NO: 68 - protein, 42 aa, African Swine fever virus
TERITYLKQIVHTIKYESGRRFLVDIIHSIYQSYSLKHEDIL

SEQ ID NO: 69 - DNA, 81 bp, African Swine fever virus
  source 1..81: mol_type = genomic DNA
gcgcaggttaaatatacccttcaagagcttatttcctactgcagcgctctaaccattttacattatgactattcaaccctt

SEQ ID NO: 70 - protein, 27 aa, African Swine fever virus
AQVKYTLQELISYCSALTILHYDYSTL

SEQ ID NO: 71 - DNA, 66 bp, African Swine fever virus
  source 1..66: mol_type = genomic DNA
gcacgaaacccctttgtatcccaaagtatgtccttgaactattacttttatgaacctgaactaagc

SEQ ID NO: 72 - protein, 22 aa, African Swine fever virus
ARNPFVSQSMSLNYYFYEPELS

SEQ ID NO: 73 - DNA, 57 bp, African Swine fever virus
  source 1..57: mol_type = genomic DNA
gtgtatgaaaagggtaagaccatgcccgtggaattttactatgaacaagagtttgat

SEQ ID NO: 74 - protein, 19 aa, African Swine fever virus
VYEKGKTMPVEFYYEQEFD

SEQ ID NO: 75 - DNA, 51 bp, African Swine fever virus
  source 1..51: mol_type = genomic DNA
attaccaaggaagaaatcatgcaagcctatgctttggagtatgccatgtat

SEQ ID NO: 76 - protein, 17 aa, African Swine fever virus
ITKEEIMQAYALEYAMY

SEQ ID NO: 77 - DNA, 2679 bp, synthetic construct
  source 1..2679: mol_type = other DNA
atgtttatgcgcgaaattaaagtaaaggaagtgttatacttttatacaatgcaggctgcccaagagggaagagttcccggtttttcaaaagaaatgctatttcaatatatacgctactttacagataatttgtgcttcatgatgcagtgcaaaagcatttataaggtgggaaacccttttcctcagatgactaaaacggaacaatttattagaaaccgcattaatttcattccgatttatgcgaaaaacgagacactggtatttgctctgcggagtttaaacaatagctgtgagattgaacagtacccaacggataaaaaagaatatatggcgcttagcggttacaagcaaagctctatgacccaaaataaccaaatagaaactattctggttcaaaaacgttacagccttgctttttcagaatttattcattgtcattactctataaatgctaatgaccgcatgtggtatcatatttggattgaaactccagtctacgaactataccacaaaaaataccaaaaatttaggaaatttaaaaaatctatgtcatactttgacggtaaaacagaatataagcatatctacttccttgcaatgttatgtaagtcgttggaggaacccgtggcccaaggtgaccatgtgcctgaccatatcaacatcctaaaaagaaaccaaatatttccgctgtttgcgcctaccccaagaggcgagggtagatttaatagcggaagaggatatatgcatgtaagattttctgctgttgtttcttacttaaatgcctttgatttaatagcggccgttaaaattattaaaaatgacagttcgcaaaataatgttgcagaagtggggcaaattgtgccggtacagcttgctaacagcagcgtgtactatatacctggcagacaacagtctaaaaaagacttcaagcagatatgcttttttgaaaaactttactatacctactctataagctcggatatgataattaacgtcatcatggatgtattttacgagacatattctttaccttataacatcaatctaacccgtgaacaaattggattaaataaaaagcgagaacttaaatactcctttcatatcatactttatacatactcagtattaaacaataatgaggccgaccaagtgatgacaaagagcatagaggttcatgagtccattctctttgaagaactgcctgatactcaaaaagaatcgatttttaatcaattcaatagcggcctgcacaaatactttgctccctcttttgccattttcatgtggatgctcgaaacggcaaattatgttatatgcttggacgcaaacctaggaaatcgaacgtataatattctacagcgttttcgcggggatgtccctttgaccaatgaacaattaatgacgaaactcgttgatgaatttgttcagtatgatttaagcgcgatcagctttgagtttaagcttaaaaagcccaataaaacggacattgatattcatgaagtacgatatggagcctacacacttttcatgtatggttccctcgaaaacggttacaaagcagaagtaaggatggggtaccgcgagaaggaaaaagagtttgcaccatacattcgaatattttttaaaagcctgtatgagcgacgaaaagccattacttacttaaataatatgggctacaacacggccgcggactcccgagaattaaaactacctcttacaagttggatacagcttcagcactattcctacgagcctcgcggcttggtaaatgttatccccgatcgcagagaggtaggaattctgtcatacacctcgctgtatgactgtatctactacgcgggaggacacaaggtatgcaatatgctcattgcctatgccatccatgatgaatacggccgtattgcttgccgggatgaggcaaatagcctcatggccaagggtgaatctcttcactacgtctcctttcactttaacaatcgtctcgtgcacgaaaaagtgcttctgtctatgaaagccatgtctacactatgcgccgaggtgaatgaatacctgcgaatggtgttaatagagtttttaacaggtttcttctatttatatggaaagagactgttttccatttgtcggaagaacattttcttccttccaaatgattttagcaagcataccctacaatggctgggattatattggaaagagcatggctccgtcctggccgtgaaaaatcaatcttccaggaaaactttgaacttgttgctatcttacataaattacaaggtgaaaaatgttaaaaagctgacagaaagaattacttatctcaaacagatagtgcacaccataaaatatgaaagtggaaggcgatttttggtagacatcattcacagcatttaccaaagttactcactaaaacacgaagatattcttgcgcaggttaaatatacccttcaagagcttatttcctactgcagcgctctaaccattttacattatgactattcaacccttgcacgaaacccctttgtatcccaaagtatgtccttgaactattacttttatgaacctgaactaagcgtgtatgaaaagggtaagaccatgcccgtggaattttactatgaacaagagtttgatattaccaaggaagaaatcatgcaagcctatgctttggagtatgccatgtattga

SEQ ID NO: 78 - protein, 892 aa, synthetic construct
MFMREIKVKEVLYFYTMQAAQEGRVPGFSKEMLFQYIRYFTDNLCFMMQCKSIYKVGNPFPQMTKTEQFIRNRINFIPIYAKNETLVFALRSLNNSCEIEQYPTDKKEYMALSGYKQSSMTQNNQIETILVQKRYSLAFSEFIHCHYSINANDRMWYHIWIETPVYELYHKKYQKFRKFKKSMSYFDGKTEYKHIYFLAMLCKSLEEPVAQGDHVPDHINILKRNQIFPLFAPTPRGEGRFNSGRGYMHVRFSAVVSYLNAFDLIAAVKIIKNDSSQNNVAEVGQIVPVQLANSSVYYIPGRQQSKKDFKQICFFEKLYYTYSISSDMIINVIMDVFYETYSLPYNINLTREQIGLNKKRELKYSFHIILYTYSVLNNNEADQVMTKSIEVHESILFEELPDTQKESIFNQFNSGLHKYFAPSFAIFMWMLETANYVICLDANLGNRTYNILQRFRGDVPLTNEQLMTKLVDEFVQYDLSAISFEFKLKKPNKTDIDIHEVRYGAYTLFMYGSLENGYKAEVRMGYREKEKEFAPYIRIFFKSLYERRKAITYLNNMGYNTAADSRELKLPLTSWIQLQHYSYEPRGLVNVIPDRREVGILSYTSLYDCIYYAGGHKVCNMLIAYAIHDEYGRIACRDEANSLMAKGESLHYVSFHFNNRLVHEKVLLSMKAMSTLCAEVNEYLRMVLIEFLTGFFYLYGKRLFSICRKNIFFLPNDFSKHTLQWLGLYWKEHGSVLAVKNQSSRKTLNLLLSYINYKVKNVKKLTERITYLKQIVHTIKYESGRRFLVDIIHSIYQSYSLKHEDILAQVKYTLQELISYCSALTILHYDYSTLARNPFVSQSMSLNYYFYEPELSVYEKGKTMPVEFYYEQEFDITKEEIMQAYALEYAMY

SEQ ID NO: 79 - DNA, 3171 bp, synthetic construct
  source 1..3171: mol_type = other DNA
atgtttatgcgcgaaattaaagtaaaggaagtgttatacttttatacaatgcaggctgcccaagagggaagagttcccggtttttcaaaagaaatgctatttcaatatatacgctactttacagataatttgtgcttcatgatgcagtgcaaaagcatttataaggtgggaaacccttttcctcagatgactaaaacggaacaatttattagaaaccgcattaatttcattccgatttatgcgaaaaacgagacactggtatttgctctgcggagtttaaacaatagctgtgagattgaacagtacccaacggataaaaaagaatatatggcgcttagcggttacaagcaaagctctatgacccaaaataaccaaatagaaactattctggttcaaaaacgttacagccttgctttttcagaatttattcattgtcattactctataaatgctaatgaccgcatgtggtatcatatttggattgaaactccagtctacgaactataccacaaaaaataccaaaaatttaggaaatttaaaaaatctatgtcatactttgacggtaaaacagaatataagcatatctacttccttgcaatgttatgtaagtcgttggaggaacccgtggcccaaggtgaccatgtgcctgaccatatcaacatcctaaaaagaaaccaaatatttccgctgtttgcgcctaccccaagaggcgagggtagatttaatagcggaagaggatatatgcatgtaagattttctgctgttgtttcttacttaaatgcctttgatttaatagcggccgttaaaattattaaaaatgacagttcgcaaaataatgttgcagaagtggggcaaattgtgccggtacagcttgctaacagcagcgtgtactatatacctggcagacaacagtctaaaaaagacttcaagcagatatgcttttttgaaaaactttactatacctactctataagctcggatatgataattaacgtcatcatggatgtattttacgagacatattctttaccttataacatcaatctaacccgtgaacaaattggattaaataaaaagcgagaacttaaatactcctttcatatcatactttatacatactcagtattaaacaataatgaggccgaccaagtgatgacaaagagcatagaggttcatgagtccattctctttgaagaactgcctgatactcaaaaagaatcgatttttaatcaattcaatagcggcctgcacaaatactttgctccctcttttgccattttcatgtggatgctcgaaacggcaaattatgttatatgcttggacgcaaacctaggaaatcgaacgtataatattctacagcgttttcgcggggatgtccctttgaccaatgaacaattaatgacgaaactcgttgatgaatttgttcagtatgatttaagcgcgatcagctttgagtttaagcttaaaaagcccaataaaacggacattgatattcatgaagtacgatatggagcctacacacttttcatgtatggttccctcgaaaacggttacaaagcagaagtaaggatggggtaccgcgagaaggaaaaagagtttgcaccatacattcgaatattttttaaaagcctgtatgagcgacgaaaagccattacttacttaaataatatgggctacaacacggccgcggactcccgagaattaaaactacctcttacaagttggatacagcttcagcactattcctacgagcctcgcggcttggtaaatgttatccccgatcgcagagaggtaggaattctgtcatacacctcgctgtatgactgtatctactacgcgggaggacacaaggtatgcaatatgctcattgcctatgccatccatgatgaatacggccgtattgcttgccgggatgaggcaaatagcctcatggccaagggtgaatctcttcactacgtctcctttcactttaacaatcgtctcgtgcacgaaaaagtgcttctgtctatgaaagccatgtctacactatgcgccgaggtgaatgaatacctgcgaatggtgttaatagagtttttaacaggtttcttctatttatatggaaagagactgttttccatttgtcggaagaacattttcttccttccaaatgattttagcaagcataccctacaatggctgggattatattggaaagagcatggctccgtcctggccgtgaaaaatcaatcttccaggaaaactttgaacttgttgctatcttacataaattacaaggtgaaaaatgttaaaaagctgacagaaagaattacttatctcaaacagatagtgcacaccataaaatatgaaagtggaaggcgatttttggtagacatcattcacagcatttaccaaagttactcactaaaacacgaagatattcttgcgcaggttaaatatacccttcaagagcttatttcctactgcagcgctctaaccattttacattatgactattcaacccttgcacgaaacccctttgtatcccaaagtatgtccttgaactattacttttatgaacctgaactaagcgtgtatgaaaagggtaagaccatgcccgtggaattttactatgaacaagagtttgatattaccaaggaagaaatcatgcaagcctatgctttggagtatgccatgtatggcggcgggggaagcatgatcagcctgatcgccgccctggccgtggactacgtgctgggcatggagaacgccatgccctggaacctgcccgccgacctggcctggttcaagcggaacaccctgaacaagcccgtgatcatgggcagacacacctgggagtccatcggcagacccctgcccggcagaaagaacatcatcctatcgtcccagccctccaccgacgaccgggtgacctgggtgaagagcgtggacgaggccatcgccgcctgcggcgacgtgcccgagatcatggtgatcggcggcggcagagtgatcgagcagttcctgcccaaggcccagaagctgtacctgacccacctggacgccgaggtggagggcgacacccacttccccgactacgagcccgacgactgggagtccgtgttcagcgagttccacgacgccgacgcccagaacagccactcctactgcttcgagatcctggagagaaggtag

SEQ ID NO: 80 - protein, 1056 aa, synthetic construct
MFMREIKVKEVLYFYTMQAAQEGRVPGFSKEMLFQYIRYFTDNLCFMMQCKSIYKVGNPFPQMTKTEQFIRNRINFIPIYAKNETLVFALRSLNNSCEIEQYPTDKKEYMALSGYKQSSMTQNNQIETILVQKRYSLAFSEFIHCHYSINANDRMWYHIWIETPVYELYHKKYQKFRKFKKSMSYFDGKTEYKHIYFLAMLCKSLEEPVAQGDHVPDHINILKRNQIFPLFAPTPRGEGRFNSGRGYMHVRFSAVVSYLNAFDLIAAVKIIKNDSSQNNVAEVGQIVPVQLANSSVYYIPGRQQSKKDFKQICFFEKLYYTYSISSDMIINVIMDVFYETYSLPYNINLTREQIGLNKKRELKYSFHIILYTYSVLNNNEADQVMTKSIEVHESILFEELPDTQKESIFNQFNSGLHKYFAPSFAIFMWMLETANYVICLDANLGNRTYNILQRFRGDVPLTNEQLMTKLVDEFVQYDLSAISFEFKLKKPNKTDIDIHEVRYGAYTLFMYGSLENGYKAEVRMGYREKEKEFAPYIRIFFKSLYERRKAITYLNNMGYNTAADSRELKLPLTSWIQLQHYSYEPRGLVNVIPDRREVGILSYTSLYDCIYYAGGHKVCNMLIAYAIHDEYGRIACRDEANSLMAKGESLHYVSFHFNNRLVHEKVLLSMKAMSTLCAEVNEYLRMVLIEFLTGFFYLYGKRLFSICRKNIFFLPNDFSKHTLQWLGLYWKEHGSVLAVKNQSSRKTLNLLLSYINYKVKNVKKLTERITYLKQIVHTIKYESGRRFLVDIIHSIYQSYSLKHEDILAQVKYTLQELISYCSALTILHYDYSTLARNPFVSQSMSLNYYFYEPELSVYEKGKTMPVEFYYEQEFDITKEEIMQAYALEYAMYGGGGSMISLIAALAVDYVLGMENAMPWNLPADLAWFKRNTLNKPVIMGRHTWESIGRPLPGRKNIILSSQPSTDDRVTWVKSVDEAIAACGDVPEIMVIGGGRVIEQFLPKAQKLYLTHLDAEVEGDTHFPDYEPDDWESVFSEFHDADAQNSHSYCFEILERR

SEQ ID NO: 81 - DNA, 568 bp, synthetic construct
  source 1..568: mol_type = other DNA
tccctcccccccccctaacgttactggccgaagccgcttggaataaggccggtgtgcgtttgtctatatgttattttccaccatattgccgtcttttggcaatgtgagggcccggaaacctggccctgtcttcttgacgagcattcctaggggtctttcccctctcgccaaaggaatgcaaggtctgttgaatgtcgtgaaggaagcagttcctctggaagcttcttgaagacaaacaacgtctgtagcgaccctttgcaggcagcggaaccccccacctggcgacaggtgcctctgcggccaaaagccacgtgtataagatacacctgcaaaggcggcacaaccccagtgccacgttgtgagttggatagttgtggaaagagtcaaatggctctcctcaagcgtattcaacaaggggctgaaggatgcccagaaggtaccccattgtatgggatctgatctggggcctcggtgcacatgctttacatgtgtttagtcgaggttaaaaaaacgtctaggccccccgaaccacggggacgtggttttcctttgaaaaacacgatgataa

SEQ ID NO: 82 - DNA, 34 bp, synthetic construct
  source 1..34: mol_type = other DNA
ataacttcgtatagcatacattatacgaagttat

SEQ ID NO: 83 - DNA, 21 bp, synthetic construct
  source 1..21: mol_type = other DNA
gacgacgacaatagtgttctg

SEQ ID NO: 84 - DNA, 19 bp, synthetic construct
  source 1..19: mol_type = other DNA
cattagatccgccaatacg

SEQ ID NO: 85 - DNA, 22 bp, synthetic construct
  source 1..22: mol_type = other DNA
tcgaggttattggttgtggatc

SEQ ID NO: 86 - DNA, 20 bp, synthetic construct
  source 1..20: mol_type = other DNA
ttagtttcctctggaagcac

SEQ ID NO: 87 - DNA, 20 bp, synthetic construct
  source 1..20: mol_type = other DNA
caaggtccctattgttacag

SEQ ID NO: 88 - DNA, 20 bp, synthetic construct
  source 1..20: mol_type = other DNA
cgtatatgtgtaccgggagc

SEQ ID NO: 89 - protein, 5 aa, synthetic construct
GGGGS

SEQ ID NO: 90 - protein, 15 aa, synthetic construct
GSAGSAAGSGEFGSG

SEQ ID NO: 91 - protein, 5 aa, synthetic construct
EAAAK

SEQ ID NO: 92 - protein, 16 aa, synthetic construct
EFPKPSTPPGSSGGAP

SEQ ID NO: 93 - protein, 7 aa, synthetic construct
KESGSVS

SEQ ID NO: 94 - protein, 14 aa, synthetic construct
EGKSSGSGSESKST

SEQ ID NO: 95 - DNA, 1032 bp, synthetic construct
  source 1..1032: mol_type = other DNA
atgtctaatctcctgacagtccaccagaatctgcccgctctccccgtggatgcaacttccgatgaggtgcggaagaatctcatggatatgtttcgcgatagacaggcttttagcgagcacacttggaagatgctcctgtccgtgtgtaggtcttgggccgcttggtgtaagctcaataaccgcaagtggttcccagccgagcccgaggatgtgcgcgactacctgctgtacctccaggctaggggactggcagtcaagactattcagcagcacctcggccagctgaacatgctccaccgccggtccggcctccctagaccatctgattccaatgccgtgtcactcgtcatgagacgcattagaaaggagaacgtcgacgctggcgagcgcgctaagcaggccctcgcctttgagcggaccgactttgatcaggtgagatccctcatggagaactctgatcggtgccaggacattcggaatctcgcctttctgggaattgcatacaacaccctcctgcgcattgcagagatcgctaggatcagagtcaaggatatttcacgcactgacggagggcgcatgctcatccacatcggacgcacaaagacactcgtgtctactgctggcgtcgagaaggctctgtcactgggagtgacaaagctggtcgagcggtggattagcgtgtccggcgtcgccgacgaccctaataattacctgttttgtagagtgcggaagaacggcgtcgctgccccttctgcaacttcacagctgtctactagggcactggagggaattttcgaggcaacccacagactcatttacggggccaaggacgatagcgggcagcggtacctggcttggtccggccactcagctagagtgggagccgcccgcgatatggctagagccggggtctctatcccagagattatgcaggcagggggatggaccaatgtgaatattgtgatgaactacatcagaaacctcgattctgagaccggggctatggtgcgcctgctcgaggacggcgattga

SEQ ID NO: 96 - protein, 343 aa, synthetic construct
MSNLLTVHQNLPALPVDATSDEVRKNLMDMFRDRQAFSEHTWKMLLSVCRSWAAWCKLNNRKWFPAEPEDVRDYLLYLQARGLAVKTIQQHLGQLNMLHRRSGLPRPSDSNAVSLVMRRIRKENVDAGERAKQALAFERTDFDQVRSLMENSDRCQDIRNLAFLGIAYNTLLRIAEIARIRVKDISRTDGGRMLIHIGRTKTLVSTAGVEKALSLGVTKLVERWISVSGVADDPNNYLFCRVRKNGVAAPSATSQLSTRALEGIFEATHRLIYGAKDDSGQRYLAWSGHSARVGAARDMARAGVSIPEIMQAGGWTNVNIVMNYIRNLDSETGAMVRLLEDGD

SEQ ID NO: 97 - DNA, 1098 bp, African swine fever virus
  source 1..1098: mol_type = genomic DNA
atgatcattctcatctttctgatcttctctaacatcgtgctctccatcgactactgggtgagcttcaacaagaccatcatcttggacagcaacatcacaaacgacaacaacgacatcaacggcgtgtcttggaacttcttcaacaacagcttcaacacactggccacttgtggaaaggccggaaacttctgcgagtgctctaactacagcacctctatctacaacatcaccaacaactgcagcctgaccatcttccctcacaacgacgtgttcgacaccacctaccaggtggtgtggaaccagatcatcaactacaccatcaagctgctgacaccagctacaccaccaaacatcacctacaactgcaccaacttcttgatcacatgcaagaagaacaacggaaccaacaccaacatctacctgaacatcaacgacaccttcgtgaagtacaccaacgagtccatcttggagtacaactggaacaactcaaacatcaacaacttcaccgccacatgcatcatcaacaacaccatcagcaccagcaacgagaccactctgatcaactgcacctacctcacactctccagcaactacttctacaccttcttcaagctgtactacatacctctcagcatcatcatcggcatcacaatcagcattctgctgatctctatcatcaccttcttgagcctgagaaagcggaagaagcacgtggaagagatcgagagtccgccacctgagagcaacgaagaagagcagtgtcagcatgatgacaccaccagcatccacgagccttctccaagagagcctctgcttccaaagccttacagccggtaccagtacaacacaccaatctactacatgagaccaagcacacagccactgaaccctttcccactgcctaagccttgtccgcctccgaaaccttgtccaccacctaagccatgtccacctccaaagccatgcccttctgcagagagctactctccaccgaaacctctgccaagcattccactgctgccaaacatccctccactgagcacacagaacatcagcctgattcacgtggatcgcatcattggaggcggtggaagctga

SEQ ID NO: 98 - protein, 365 aa, African swine fever virus
MIILIFLIFSNIVLSIDYWVSFNKTIILDSNITNDNNDINGVSWNFFNNSFNTLATCGKAGNFCECSNYSTSIYNITNNCSLTIFPHNDVFDTTYQVVWNQIINYTIKLLTPATPPNITYNCTNFLITCKKNNGTNTNIYLNINDTFVKYTNESILEYNWNNSNINNFTATCIINNTISTSNETTLINCTYLTLSSNYFYTFFKLYYIPLSIIIGITISILLISIITFLSLRKRKKHVEEIESPPPESNEEEQCQHDDTTSIHEPSPREPLLPKPYSRYQYNTPIYYMRPSTQPLNPFPLPKPCPPPKPCPPPKPCPPPKPCPSAESYSPPKPLPSIPLLPNIPPLSTQNISLIHVDRIIGGGGS

SEQ ID NO: 99 - DNA, 22 bp, synthetic construct
  source 1..22: mol_type = other DNA
gaacatacagtttgcactcatg

SEQ ID NO: 100 - DNA, 22 bp, synthetic construct
  source 1..22: mol_type = other DNA
cgcatactatatgcgatgattg